European Patent Specification EP 3 862 010 B1, published May 7, 2025. Title: USE OF AKKERMANSIA FOR TREATING METABOLIC DISORDERS. Applicant: Université catholique de Louvain Wageningen Universiteit CANI, Patrice. The sequence listing filed with the application follows.

SEQUENCE LISTING (30 sequences)

SEQ ID NO: 1 - DNA, 23 bp, Artificial Sequence
  source 1..23: /mol_type="unassigned DNA" /note="Primer RPL-19 Forward" /organism="Artificial Sequence"
gaaggtcaaagggaatgtgttca

SEQ ID NO: 2 - DNA, 16 bp, Artificial Sequence
  source 1..16: /mol_type="unassigned DNA" /note="Primer RPL-19 Reverse" /organism="Artificial Sequence"
cctgttgctcacttgt

SEQ ID NO: 3 - DNA, 21 bp, Artificial Sequence
  source 1..21: /mol_type="unassigned DNA" /note="Primer Reg3g Forward" /organism="Artificial Sequence"
ttcctgtcctccatgatcaaa

SEQ ID NO: 4 - DNA, 20 bp, Artificial Sequence
  source 1..20: /mol_type="unassigned DNA" /note="Primer Reg3g Reverse" /organism="Artificial Sequence"
catccacctctgttgggttc

SEQ ID NO: 5 - DNA, 27 bp, Artificial Sequence
  source 1..27: /mol_type="unassigned DNA" /note="Primer Lyz1 Forward" /organism="Artificial Sequence"
gccaaggtctacaatcgttgtgagttg

SEQ ID NO: 6 - DNA, 23 bp, Artificial Sequence
  source 1..23: /mol_type="unassigned DNA" /note="Primer Lyz1 Reverse" /organism="Artificial Sequence"
cagtcagccagcttgacaccacg

SEQ ID NO: 7 - DNA, 22 bp, Artificial Sequence
  source 1..22: /mol_type="unassigned DNA" /note="Primer Pla2g2a Forward" /organism="Artificial Sequence"
aggattcccccaaggatgccac

SEQ ID NO: 8 - DNA, 25 bp, Artificial Sequence
  source 1..25: /mol_type="unassigned DNA" /note="Primer Pla2g2a Reverse" /organism="Artificial Sequence"
cagccgtttctgacaggagttctgg

SEQ ID NO: 9 - DNA, 24 bp, Artificial Sequence
  source 1..24: /mol_type="unassigned DNA" /note="Primer CD11cc Forward" /organism="Artificial Sequence"
acgtcagtacaaggagatgttgga

SEQ ID NO: 10 - DNA, 26 bp, Artificial Sequence
  source 1..26: /mol_type="unassigned DNA" /note="Primer CD11cc Reverse" /organism="Artificial Sequence"
atcctattgcagaatgcttctttacc

SEQ ID NO: 11 - DNA, 26 bp, Artificial Sequence
  source 1..26: /mol_type="unassigned DNA" /note="Primer Defa Forward" /organism="Artificial Sequence"
ggtgatcatcagaccccagcatcagt

SEQ ID NO: 12 - DNA, 24 bp, Artificial Sequence
  source 1..24: /mol_type="unassigned DNA" /note="Primer Defa Reverse" /organism="Artificial Sequence"
aagagactaaaactgaggagcagc

SEQ ID NO: 13 - DNA, 20 bp, Artificial Sequence
  source 1..20: /mol_type="unassigned DNA" /note="Primer Fasn Forward" /organism="Artificial Sequence"
ttccaagacgaaaatgatgc

SEQ ID NO: 14 - DNA, 20 bp, Artificial Sequence
  source 1..20: /mol_type="unassigned DNA" /note="Primer Fasn Reverse" /organism="Artificial Sequence"
aattgtgggatcaggagagc

SEQ ID NO: 15 - DNA, 24 bp, Artificial Sequence
  source 1..24: /mol_type="unassigned DNA" /note="Primer Cpt1a Forward" /organism="Artificial Sequence"
agaccgtgaggaactcaaacctat

SEQ ID NO: 16 - DNA, 18 bp, Artificial Sequence
  source 1..18: /mol_type="unassigned DNA" /note="Primer Cpt1a Reverse" /organism="Artificial Sequence"
tgaagagtcgctcccact

SEQ ID NO: 17 - DNA, 22 bp, Artificial Sequence
  source 1..22: /mol_type="unassigned DNA" /note="Primer Pgc1a Forward" /organism="Artificial Sequence"
agccgtgaccactgacaacgag

SEQ ID NO: 18 - DNA, 23 bp, Artificial Sequence
  source 1..23: /mol_type="unassigned DNA" /note="Primer Pgc1a Reverse" /organism="Artificial Sequence"
gctgcatggttctgagtgctaag

SEQ ID NO: 19 - DNA, 19 bp, Artificial Sequence
  source 1..19: /mol_type="unassigned DNA" /note="Primer Ppara Forward" /organism="Artificial Sequence"
caacggcgtcgaagacaaa

SEQ ID NO: 20 - DNA, 19 bp, Artificial Sequence
  source 1..19: /mol_type="unassigned DNA" /note="Primer Ppara Reverse" /organism="Artificial Sequence"
tgacggtctccacggacat

SEQ ID NO: 21 - DNA, 21 bp, Artificial Sequence
  source 1..21: /mol_type="unassigned DNA" /note="Primer Acox1 Forward" /organism="Artificial Sequence"
ctatgggatcagccagaaagg

SEQ ID NO: 22 - DNA, 21 bp, Artificial Sequence
  source 1..21: /mol_type="unassigned DNA" /note="Primer Acox1 Reverse" /organism="Artificial Sequence"
agtcaaaggcatccaccaaag

SEQ ID NO: 23 - DNA, 23 bp, Artificial Sequence
  source 1..23: /mol_type="unassigned DNA" /note="Primer Acc1 Forward" /organism="Artificial Sequence"
tgttgagacgctggtttgtagaa

SEQ ID NO: 24 - DNA, 25 bp, Artificial Sequence
  source 1..25: /mol_type="unassigned DNA" /note="Primer Acc1 Reverse" /organism="Artificial Sequence"
ggtccttattattgtcccagacgta

SEQ ID NO: 25 - DNA, 21 bp, Artificial Sequence
  source 1..21: /mol_type="unassigned DNA" /note="Primer Cebpa Forward" /organism="Artificial Sequence"
gagccgagataaagccaaaca

SEQ ID NO: 26 - DNA, 16 bp, Artificial Sequence
  source 1..16: /mol_type="unassigned DNA" /note="Primer Cebpa Reverse" /organism="Artificial Sequence"
gcgcaggcggtcattg

SEQ ID NO: 27 - DNA, 20 bp, Artificial Sequence
  source 1..20: /mol_type="unassigned DNA" /note="Primer G6pc Forward" /organism="Artificial Sequence"
aggaaggatggaggaaggaa

SEQ ID NO: 28 - DNA, 20 bp, Artificial Sequence
  source 1..20: /mol_type="unassigned DNA" /note="Primer G6pc Reverse" /organism="Artificial Sequence"
tggaaccagatgggaaagag

SEQ ID NO: 29 - DNA, 20 bp, Artificial Sequence
  source 1..20: /mol_type="unassigned DNA" /note="Primer F-Akkermansia muciniphila" /organism="Artificial Sequence"
ccttgcggttggcttcagat

SEQ ID NO: 30 - DNA, 20 bp, Artificial Sequence
  source 1..20: /mol_type="unassigned DNA" /note="Primer R-Akkermansia muciniphila" /organism="Artificial Sequence"
cagcacgtgaaggtggggac